European Patent Application EP 4 151 718 A1, published March 22, 2023. Title: Genetically Engineered Microorganism and Method of Producing Organic Acids. Applicant: Toray Industries, Inc. The sequence listing filed with the application follows.

SEQUENCE LISTING (50 sequences)

SEQ ID NO: 1 - protein, 109 aa, Escherichia coli MG1655
METTKPSFQDVLEFVRLFRRKNKLQREIQDVEKKIRDNQKRVLLLDNLSDYIKPGMSVEAIQGIIASMKGDYEDRVDDYIIKNAELSKERRDISKKLKAMGEMKNGEAK

SEQ ID NO: 2 - protein, 107 aa, Serratia grimesii NBRC13537
MKMDNANKPSFQDVLEFVRMFRRKNKLQREIIDNEKKVRDNQKRVLLLDNLSEYIKPGMSIEDVQGIIGNMRSDYEDRVDDYIIKNADLSKERRELSKKLKAMGEVK

SEQ ID NO: 3 - protein, 94 aa, Acinetobacter baumannii
FRRKNKLQREIQDIEKKIRDNQKRVLLLDNLSDYIKPGMSVEAIQGIIASMKSDYEDRVDDYIIKNAEISKERRDISKKLKAMGEMKHADVKAE

SEQ ID NO: 4 - protein, 114 aa, Actinobacillus succinogenes 130Z
MENVNKQSFQEVLEYVRINRQRNKLLREIGDCERKIRDNKKRVLLLDNLTDYIQDNMTIEDIRAIINNMHDDYENRVDDYVIKAAELSKQRRDLKTRMKELKASHAALAKKGKE

SEQ ID NO: 5 - protein, 111 aa, Aerobacter cloacae
METTKPSFQDVLEFVRLFRRKNKLQREIQDVEKKIRDNQKRVLLLDNLSDYIKPGMSVEAIQGIIASMKSDYEDRVDDYIIKNAELSKERRDISKKLKVMGEIKNGEAKGE

SEQ ID NO: 6 - protein, 114 aa, Basfia succiniciproducens
MENVNKQSFQDVLEYVRLYRLRNKLLRDIGDNDRKIRDNQKRVLLLDNLSQYITNDMSVEDIRAIIENMRDDYEGRVDDYMIRNADLSKERREIKEKMKAQKKAHAELLKKADD

SEQ ID NO: 7 - protein, 107 aa, Hafnia paralvei
MENVNKPTFQNVLEFVRMFRRKNKLQREIVDNEKKIRDNQKRVLLLDNLSEYIKPGMSVEAIQAIIADMRGNYEDRVDDYIIKNADLSKERRELSKKLKALGEGESK

SEQ ID NO: 8 - protein, 107 aa, Pseudomonas aeruginosa
METTKPSFQDVLEFVRLYRRKNKLQREIQDVEKKIRDNQKRVLLLDNLSDYIKPGMSVEAIQGIIASMKSDYEDRVDDYIIKNAELSKERRDISKKLKVMGEAKVEG

SEQ ID NO: 9 - protein, 112 aa, Shimwellia blattae
MENTKPSFQDVLEFVRLFRRKNKLQREIQDVEKKIRDNQKRVLLLDNLSDYIKPGMTVEAIQGIIASMKSDYEDRVDDYIIKNAELSKERRDISKKLKVMGEMKNQDPEAKA

SEQ ID NO: 10 - DNA, 330 bp, Escherichia coli MG1655
atggaaactaccaagccttcattccaggacgtactggaatttgttcgtctgttccgtcgtaagaacaaactgcaacgtgaaattcaggacgttgagaaaaagatccgtgacaaccagaagcgcgtcctgctgctggacaacctgagcgattacatcaagccggggatgagcgttgaagcaatccagggcatcatcgccagcatgaaaggtgactatgaagatcgcgttgacgattacatcatcaaaaatgccgagctctccaaagaacgccgcgatatctccaaaaagctgaaagctatgggcgaaatgaaaaacggcgaagcgaagtaa

SEQ ID NO: 11 - DNA, 324 bp, Serratia grimesii NBRC13537
atgaagatggataatgcaaataagccgagtttccaggacgttctggagtttgtgcgtatgttccgccgtaaaaataagctgcaacgcgaaattatcgacaacgaaaagaaagttcgtgataaccaaaagcgtgtgctgctactcgacaacctgagtgagtacatcaagccaggcatgagcattgaagacgttcagggcatcattggcaacatgcgcagcgactatgaagatcgcgttgatgactacatcatcaaaaatgccgatctgtctaaagaacgtcgcgaactgtccaaaaagctgaaagctatgggcgaagtgaagtaa

SEQ ID NO: 12 - protein, 107 aa, Artificial Sequence
  Synthetic peptide
MKMDNANKPSFQDVLEFVRMFRRKNKLQREIIDNEKKVRDNQKRVLLLDNLSEYIKPGMSIEDVQGIIGNMRSDYEDRVDDYIIKNVDLSKERRELSKKLKAMGEVK

SEQ ID NO: 13 - DNA, 774 bp, Pseudomonas putida KT2440
atgccgcgatatatcgatgtgcaggcgcccgaacatggcgttcagctcattaccctgcaacggcccgaggccttgaatgccctgtgcaccgagctactggcagaactggccgctgcgctgcaggctgccgggaacgacgagcatgtccgtgccacagtgattaccggcagcgccaaggcattcgccgcaggcgccgacatccgcgagatggccgatcgcgacctggtcggcatcctcaatgacccgcgcgtagcgcattggcaaagcatcgccgcattcgccaaaccgctgattgctgcagtcaacggctatgccctgggtggcggttgcgaactggcaatgtgcgccgacatcgtcatcgccagtaccgacgcccgtttcggccagccggaaatcaaccttggcatcatccccggtgctggcggcacccagcgcctgttacgtgccgtcggtaagccgttggccatgcagatggtgctgacgggggaagccatcactgccctccgcgcccagcaggccggcctggtcagcgaaatcacccagcccgaactcaccgtagaacgcgccatgcaggttgcccgcagcatcgccgccaaagcgccgctggctgtgcgcctggccaaggaggcgttactgaaggccggtgataccgacctggccagcggcctgcgcttcgagcgccatgccttcaccctgctggcgggcaccgccgaccgcgatgaaggcatccgcgccttccaggaaaagcgccaggcccgcttccaagggcgctga

SEQ ID NO: 14 - DNA, 1530 bp, Serratia marcescens ATCC13880
atggcagaaagtaatgcggcaattcaatcggctgcgattatcggcgcgggaacgatgggcagaggcatcgcttatcttttcgcgcaaaaaggcattcgcacggtgctttataatcgcaacggcaataccctcaatcaggctcgcgaatatatcgcgcaagacctgaacaagaaagtcgaacagggcaagatcgcgctgcaggataaaggcgcggtgctggccaatctaatgttcacttcagtgtttgaggccatcgccgacagcgagctggtgatagaaaccatcgccgagcaagaacaaaccaaacttgaggtgctggcggccatcgccgcggtggtcaagcccgacacgctgatcgccaccaatacctcctcactgtcgcttaacaagctggctactgcggtgacgcacagcgaacgctttatcggtttgcattttttcaaccccgcgccgctgatgaagctgattgaaatcattccggcctactttaccgcgcacgccaccaccgaacgctgccgccaactggtggcggcgttggggaaacacgatgtcgtctgccaggccacgccggggttcatcgtcaatcgcatggcccgcccctactacctggaagggttccgcctgttggaagaacacgtggcgcgcgcggctcagatcgaccgcgccctcaaggccggcgggcgcttccgcatggggccgctcgagctgaccgattttatcggccaagacatcaactatcaggtcagtcggcaaatctggcaggatatgcaatacgacccgcgctatacccccggtcatctgcagcgttcactggtcgatgccggtctgttggggaaaaagaacggccgctcctattttgccgccgaagaaaccgccccgccggtgacggccgccagcaatgcagacgtcgagacgctgcgcgtttacggcgagcaccctttttttaccctgttacagcagcgagccgcgcttcagtggccacagctgcgcgtggaacaacggccggcattaccggggctggggtcggccgtccagatcaatgacgctttcaccgtcagcatcaccgatggccgcacggcgagccaactggccgagcagacggcagcggatgcctttgtggtcgatgtcgccctgaactacgccgacacgacgtatctggcggcggcgcacagccgccacgcctctgcggccaataaggcgctgtttttacgcctgctgcacacggcaatcccgcaggttgaatttatcaaggactctccggcgcttatcgtcgcccgcgtcctcagcagcctgatcaatgagtcggtgatcatggtggaaagcggcgtctgcagccgggaagacatcgatgtcgccgccgtcgcgggcgttaactacgccggcggcattttcgactggctcggcaaactgggggagaaaaacgtcaggacaacgctgagcaatctggctcagctgctgcacgcggcgcgctatgcgccgcattacacccttctgcacgccgcgcaaccggcgctgacgaccacgccttaa

SEQ ID NO: 15 - DNA, 774 bp, Pseudomonas putida KT2440; identical to SEQ ID NO: 13

SEQ ID NO: 16 - DNA, 1155 bp, Acinetobacter baylyi ADP1
atgattcgcgatgaagggatgttgcaacaattactttcgacaatacgagattttgtaaaaaatgaattgattcctcgagagcatgaagttgcagaaaaggattgtattcctgaagatattattcagcaaatgcgagaactaggcctatttggtttaaccattcccgaagaatacggtggacttggaatcacaatggaagaagaggtgaatgtcgcgtttgaacttggtcagacatccccagcatttcgttcattgattggcacaaataatggcattggttcaagtggtttaatcattgatggaactgaggagcaaaaacagaaatatttgccacgttatgccagtggagaaattattggttcattttgcttaactgaaccagaagcgggttcagatgctgcctctttaaaaacgacagcggtaaaagatggtgatttctacatattaaatggaaccaagcgttttattaccaatgcaccgcatgcagcaacatttaccgtaatggcacgcaccaatccagcaattaaaggggcaggtggaatttctgcttttttggtagaagccaatacaccaggtatcacactaggcaaaatagatcagaaaatgggacaaaaaggctctcatacctgtgatgtgatttttgaaaattgtcgagtacctgcatctgcattaattggtggcgttgaaggcgttggttttaaaacagcaatgaaagtgctggataaaggccgtctacatattggtgcatatagtgtaggtgttgcagagcgtatgttgaatgatgcactacattatgctgtcgagcgtaagcagtttggtcaacccattgcaaattttcaattgattcaagccatgctggcagactctaaagccgaaatttatgcggctaaatgtatggttttggatgcagcacgtcgccgtgatgaaggccaaaatattagtacagaagcctcatgtgccaagatgtttgcaacagaaatgtgtggtcgagtcgcagatcgctgtgtgcaaattcatggtggggcaggttacatcagtgaatattcgattgagcgtttttatcgtgacgtgcgtttattccgtctttatgagggtacgacccaagttcagcaaattattattgccaaaaatatgattaaggaagtgacgtcctaa

SEQ ID NO: 17 - DNA, 696 bp, Pseudomonas putida KT2440
ttgatcaataaaacgtacgagtccatcgccagcgcggtggaagggattaccgacggttcgaccatcatggtcggtggcttcggcacggctggcatgccgtccgagctgatcgatggcctcattgccaccggtgcccgcgacctgaccatcatcagcaacaacgccggcaacggcgagatcggcctggccgccctgctcatggcaggcagcgtgcgcaaggtggtctgctcgttcccgcgccagtccgactcctacgtgttcgacgaactgtaccgcgccggcaagatcgagctggaagtggtcccgcagggcaacctggccgagcgtatccgcgccgcaggctccggcattggtgcgttcttctcgccaaccggctacggcaccctgctggccgagggcaaggaaacccgtgagatcgatggccgcatgtacgtgctggaaatgccgctgcacgccgacttcgcactgatcaaggcgcacaagggtgaccgttggggcaacctgacctaccgcaaggccgcccgcaacttcggcccgatcatggccatggctgccaagaccgccatcgcccaggtcgaccaggtcgtcgaactcggtgaactggacccggaacacatcatcaccccgggtatcttcgtccagcgcgtggtcgccgtcaccggtgctgccgcttcttcgattgccaaagctgtctga

SEQ ID NO: 18 - DNA, 642 bp, Pseudomonas putida KT2440
atgaccatcaccaaaaagctctcccgcaccgagatggcccaacgcgtggccgcagacatccaggaaggcgcgtacgtaaacctgggcatcggcgcaccgaccctggtggccaactacctgggcgacaaggaagtgttcctgcacagcgagaacggcctgctgggcatgggcccaagccctgcgccgggcgaggaagacgatgacctgatcaacgccggcaagcagcacgtcaccctgctgaccggtggtgccttcttccaccatgccgattcgttctcgatgatgcgtggcggccacctggacatcgctgtactgggcgccttccaggtgtcggtcaagggcgacctggccaactggcacacgggtgccgaaggctcgatcccggccgtaggcggtgcaatggacctggccaccggcgcccgccaggtgttcgtgatgatggaccacctgaccaagaccggcgaaagcaagctggtgcccgagtgcacctacccgctgaccggtatcgcttgcgtcagccgcatctacaccgacctggccgtactggaagtgacacctgaagggctgaaagtggtcgaaatctgcgcggacatcgactttgacgagctgcagaaactcagtggcgtgccgctgatcaagtga

SEQ ID NO: 19 - DNA, 4998 bp, Artificial Sequence
  Synthetic DNA fragment
ttggttgaacgctttttggcttaatggccttttgaacaccacaacactgaggaaaatgaaatgaaaacaaaaagtagcctggttttattgctgccactggcgttaagtttcgcggcctttggtggagagttcagcggcaaagtcattaagctgggcgtcgaccccacctatccgccgttggaatacaagactccacagggtgcgctgaccggattcggtgtcgatattgcgcaggcaatgtgcgatcaaatgcaggccaaatgcatttgggtcgaaagcagttgggatgggatgatcccggggttgcaggcaaaaaagtttgacgccattgcctcgtccatgaccattacgccgcagcgtcaggcgcaaatagccttctcggataaagtgtccaatgccccggcacggttggtagcccgtaaaggcagcgatctgcaacctaccgcggcttcgctgaaaggcaaatccgttggcgtacaacagggatccagccaggaagcttacgccaacgcgctatggcgaccagctggggtcaatgtggtgtcctaccaaagccagcaggaagccaatgaagatttggtcaatggacggttggatgcgtcactgttggccagtgtcagcgccagtgagtttttccatacgcctgccgggaaggattttgcctttaccggtgctgagctcaatgacagcaaatatttcggtatcggcgacggtattgggttgcgtaaagaggatacggcattgctcaatgcatttaatgccgcgctgaaagcgatcatcgccaacggcacttataagaaagtgaacgataaatactttgattttgacgtgtatggttcagggcaataagatcctttttaacccatcacatatacctgccgttcactattatttagtgaaatgagatattatgatattttctgaattgtgattaaaaaggcaactttatgcccatgcaacagaaactataaaaaatacagagaatgaaaagaaacagatagattttttagttctttaggcccgtagtctgcaaatccttttatgattttctatcaaacaaaagaggaaaatagaccagttgcaatccaaacgagagtctaatagaatgaggtcgaaaagtaaatcgcgcgggtttgttactgataaagcaggcaagacctaaaatgtgtaaagggcaaagtgtatactttggcgtcaccccttacatattttaggtctttttttattgtgcgtaactaacttgccatcttcaaacaggagggctggaagaagcagaccgctaacacagtacataaaaaaggagacatgaacgatgaacatcaaaaagtttgcaaaacaagcaacagtattaacctttactaccgcactgctggcaggaggcgcaactcaagcgtttgcgaaagaaacgaaccaaaagccatataaggaaacatacggcatttcccatattacacgccatgatatgctgcaaatccctgaacagcaaaaaaatgaaaaatatcaagttcctgaattcgattcgtccacaattaaaaatatctcttctgcaaaaggcctggacgtttgggacagctggccattacaaaacgctgacggcactgtcgcaaactatcacggctaccacatcgtctttgcattagccggagatcctaaaaatgcggatgacacatcgatttacatgttctatcaaaaagtcggcgaaacttctattgacagctggaaaaacgctggccgcgtctttaaagacagcgacaaattcgatgcaaatgattctatcctaaaagaccaaacacaagaatggtcaggttcagccacatttacatctgacggaaaaatccgtttattctacactgatttctccggtaaacattacggcaaacaaacactgacaactgcacaagttaacgtatcagcatcagacagctctttgaacatcaacggtgtagaggattataaatcaatctttgacggtgacggaaaaacgtatcaaaatgtacagcagttcatcgatgaaggcaactacagctcaggcgacaaccatacgctgagagatcctcactacgtagaagataaaggccacaaatacttagtatttgaagcaaacactggaactgaagatggctaccaaggcgaagaatctttatttaacaaagcatactatggcaaaagcacatcattcttccgtcaagaaagtcaaaaacttctgcaaagcgataaaaaacgcacggctgagttagcaaacggcgctctcggtatgattgagctaaacgatgattacacactgaaaaaagtgatgaaaccgctgattgcatctaacacagtaacagatgaaattgaacgcgcgaacgtctttaaaatgaacggcaaatggtacctgttcactgactcccgcggatcaaaaatgacgattgacggcattacgtctaacgatatttacatgcttggttatgtttctaattctttaactggcccatacaagccgctgaacaaaactggccttgtgttaaaaatggatcttgatcctaacgatgtaacctttacttactcacacttcgctgtacctcaagcgaaaggaaacaatgtcgtgattacaagctatatgacaaacagaggattctacgcagacaaacaatcaacgtttgcgccaagcttcctgctgaacatcaaaggcaagaaaacatctgttgtcaaagacagcatccttgaacaaggacaattaacagttaacaaataaaaacgcaaaagaaaatgccgatatcctattggcattttcttttatttcttatcaacataaaggtgaatcccatatgaactatataaaagcaggcaaatggctaaccgtattcctaacctttttaggaatattgctgtttatcgacttgtcgactctagaggatcctgtgtaggctggagctgcttcgaagttcctatactttctagagaataggaacttcggaataggaacttcaagatcccctcacgctgccgcaagcactcagggcgcaagggctgctaaaggaagcggaacacgtagaaagccagtccgcagaaacggtgctgaccccggatgaatgtcagctactgggctatctggacaagggaaaacgcaagcgcaaagagaaagcaggtagcttgcagtgggcttacatggcgatagctagactgggcggttttatggacagcaagcgaaccggaattgccagctggggcgccctctggtaaggttgggaagccctgcaaagtaaactggatggctttcttgccgccaaggatctgatggcgcaggggatcaagatctgatcaagagacaggatgaggatcgtttcgcatgattgaacaagatggattgcacgcaggttctccggccgcttgggtggagaggctattcggctatgactgggcacaacagacaatcggctgctctgatgccgccgtgttccggctgtcagcgcaggggcgcccggttctttttgtcaagaccgacctgtccggtgccctgaatgaactgcaggacgaggcagcgcggctatcgtggctggccacgacgggcgttccttgcgcagctgtgctcgacgttgtcactgaagcgggaagggactggctgctattgggcgaagtgccggggcaggatctcctgtcatctcaccttgctcctgccgagaaagtatccatcatggctgatgcaatgcggcggctgcatacgcttgatccggctacctgcccattcgaccaccaagcgaaacatcgcatcgagcgagcacgtactcggatggaagccggtcttgtcgatcaggatgatctggacgaagagcatcaggggctcgcgccagccgaactgttcgccaggctcaaggcgcgcatgcccgacggcgaggatctcgtcgtgacccatggcgatgcctgcttgccgaatatcatggtggaaaatggccgcttttctggattcatcgactgtggccggctgggtgtggcggaccgctatcaggacatagcgttggctacccgtgatattgctgaagagcttggcggcgaatgggctgaccgcttcctcgtgctttacggtatcgccgctcccgattcgcagcgcatcgccttctatcgccttcttgacgagttcttctgagcgggactctggggttcgaaatgaccgagatacaggtttgtggcggtcaggcacaacactcatcgccctatcttactcactttgctgtccggacaaaaacccgaagcgcctgcttcatgatctgaccccctattcgcgcccggtagcagtacagaccttgagcaggtcgcccagttcttccagttgttgtgtcagctccatgctcagccagacataaccgtaaattggcgcttcgccgtgctgactgacactggcttcctgcatcagcgttttcagttcagcggcgatttcgcttagctcgcctgccacgacagattgttgcgcttgtgggccattacgcatcgtgtccgccaatgattcaagcgaccgcagcgtcagcaattgcgcactgcgcagggttttcgcattcagcataatgaaatgggtttcacgcgaggcccaataagcgtccgccaacagctccagagtacagaccagattgcggctcaacgtttgtaccgcttcaaatacagccggaggaatatgggtttctttactgctgggaacaatcaggccgcgcaatttgaccacctgattcaagagatctttcaactgcggttccaaccgcggccgctctatcatgttcggtgacaaataagcaccgtagattttactcgcgctttgcaagcaatccgccatctgcatacgccacagaatgtaggcgcgctgagggtaaatgctggtgaacaacaacgccagcaacgaaccaaaaattacgtcaccactgcgccacaacgcggtatgcatgtcacctgcccccgcgccacaaaccaccgccagtgtaatccccaccaacagtgccatatagggccgcttaccgagtgtcagatagccgc

SEQ ID NO: 20 - DNA, 20 bp, Artificial Sequence
  Primer
ttggttgaacgctttttggc

SEQ ID NO: 21 - DNA, 18 bp, Artificial Sequence
  Primer
gcggctatctgacactcg

SEQ ID NO: 22 - DNA, 200 bp, Escherichia coli str. K-12 substr. MG1655
cgtaattgccctttaaaattcggggcgccgaccccatgtggtctcaagcccaaaggaagagtgaggcgagtcagtcgcgtaatgcttaggcacaggattgatttgtcgcaatgattgacacgattccgcttgacgctgcgtaaggtttttgtaattttacaggcaaccttttattcactaacaaatagctggtggaatat

SEQ ID NO: 23 - DNA, 30 bp, Artificial Sequence
  Primer
taccgtcgacctcgacgtaattgcccttta

SEQ ID NO: 24 - DNA, 41 bp, Artificial Sequence
  Primer
ggccccccctcgagtcattaagtactatattccaccagcta

SEQ ID NO: 25 - DNA, 32 bp, Artificial Sequence
  Primer
ctggtggaatatatgcacgacgtattcatctg

SEQ ID NO: 26 - DNA, 41 bp, Artificial Sequence
  Primer
ctcgagtcattaagtgttaactcaaacccgctcgatggcca

SEQ ID NO: 27 - DNA, 55 bp, Artificial Sequence
  Primer
gagcgggtttgagttcaattgtagctggtggaatatttgatcaataaaacgtacg

SEQ ID NO: 28 - DNA, 34 bp, Artificial Sequence
  Primer
gagtcattaagtgtttcacttgatcagcggcacg

SEQ ID NO: 29 - DNA, 35 bp, Artificial Sequence
  Primer
ctggtggaatatagtactatggcagaaagtaatgc

SEQ ID NO: 30 - DNA, 39 bp, Artificial Sequence
  Primer
ttccaccagctaagtgctagcttaaggcgtggtcgtcag

SEQ ID NO: 31 - DNA, 40 bp, Artificial Sequence
  Primer
cggccagtgaattcgagctccgtaattgccctttaaaatt

SEQ ID NO: 32 - DNA, 41 bp, Artificial Sequence
  Primer
gatccccgggtaccgcatgctatattccaccagctatttgt

SEQ ID NO: 33 - DNA, 34 bp, Artificial Sequence
  Primer
gctggtggaatatagatgccgcgatatatcgatg

SEQ ID NO: 34 - DNA, 34 bp, Artificial Sequence
  Primer
attacgccaagcttgtcagcgcccttggaagcgg

SEQ ID NO: 35 - DNA, 50 bp, Artificial Sequence
  Primer
gggcgctgacaagcttagctggtggaatatatgattcgcgatgaagggat

SEQ ID NO: 36 - DNA, 36 bp, Artificial Sequence
  Primer
tgattacgccaagcttttaggacgtcacttccttaa

SEQ ID NO: 37 - DNA, 324 bp, Artificial Sequence
  Synthetic DNA fragment
atgaagatggataatgcaaataagccgagtttccaggacgttctggagtttgtgcgtatgttccgccgtaaaaataagctgcaacgcgaaattatcgacaacgaaaagaaagttcgtgataaccaaaagcgtgtgctgctactcgacaacctgagtgagtacatcaagccaggcatgagcattgaagacgttcagggcatcattggcaacatgcgcagcgactatgaagatcgcgttgatgactacatcatcaaaaatgtcgatctgtctaaagaacgtcgcgaactgtccaaaaagctgaaagctatgggcgaagtgaagtaa

SEQ ID NO: 38 - DNA, 50 bp, Artificial Sequence
  Primer
aaatagctggtggaatatagcatgcatgaagatggataatgcaaataagc

SEQ ID NO: 39 - DNA, 46 bp, Artificial Sequence
  Primer
cgactctagaggatccccgggtaccttacttcacttcgcccatagc

SEQ ID NO: 40 - protein, 477 aa, Serratia grimesii NBRC13537
MFKNAFANLQKVGKSLMLPVSVLPIAGILLGVGSANFSWLPAVVSHVMAEAGGSVFANMPLIFAIGVALGFTNNDGVSALAAVVAYGIMVKTMAVVAPLVLHLPAEEIAAKHLADTGVLGGIISGSIAAYMFNRFFRIQLPEYLGFFAGKRFVPIISGLAAIVLGVVLSFIWPPIGTAIQTFSQWAAYQNPVVAFGIYGVVERALVPFGLHHIWNVPFQMQIGEYTNAAGQVFHGDIPRYMAGDPTAGKLSGGFLFKMYGLPAAAIAIWHSAKPENRAKVGGIMISAALTSFLTGITEPIEFSFMFVAPILYAIHAILAGLAFPICILLGMRDGTSFSHGLIDFIVLSGNSSKIWLFPIVGIIYGLVYYTIFRVLIAKLDLKTPGREDTVSEQVAQGGSEMSAALVQAFGGKENITNLDACITRLRVSVADVSKVDQAGLKKLGAAGVVVAGSGVQAIFGTKSDNLKTDMDEYIRNH

SEQ ID NO: 41 - protein, 470 aa, Serratia grimesii NBRC13537
MKKTKIVCTIGPKTESEEMLTNLLNAGMNVMRLNFSHGDYEEHGNRIKNMRAVMAKTGQNAGILLDTKGPEIRTMKLEGGKDAALVAGQTFTFTTDQSVIGNNERVAVTYAGFSADLKIGNTVLVDDGLIGMEVTNVTENEVVCKVLNSGDLGENKGVNLPGVSIQLPALAEKDKRDLIFGCEQGVDFVAASFIRKRSDVLEIREHLKAHGGEQIQIISKIENQEGLNNFDEILEASDGIMVARGDLGVEIPVEEVIFAQKMMIEKCNRARKVVITATQMLDSMIKNPRPTRAEAGDVANAILDGTDAVMLSGESAKGKYPLEAVTIMATICERTDRVMPSRIDSLNDNRKLRITEAVCRGAVETAEKLDAPLIVVATSGGKSAKSVRKYFPNAVILALTTNEVTAHQLILSKGVIPQMVKEIASTDDFYRIGKEAALASGLAQKGDVVVMVSGALVPSGTTNTASVHVL

SEQ ID NO: 42 - protein, 480 aa, Serratia grimesii NBRC13537
MSRRLRRTKIVTTLGPATDRDNNLEKIIAAGANVVRLNFSHGSAEDHQARADKVREIAAKLGRHVAILGDLQGPKIRVSTFKEGKIFLNIGDKFLLDANMSKGEGDKEKVGIDYKGLPADVVPGDVLLLDDGRVQLKVLEVQGMKVFTEVTVGGPLSNNKGINKLGGGLSAEALTEKDKADIVTAAKIGVDYLAVSFPRTGEDLNYARRLARDAGCNAKIVSKVERAEAVCSDEAMDDIILASDVVMVARGDLGVEIGDPELVGIQKKLIRRARTLNRAVITATQMMESMITNPMPTRAEVMDVANAVLDGTDAVMLSAETAAGQYPAETVAAMARVCLGAEKIPSINVSKHRLDVQFDNIEEAIAMSSMYAANHLKGVTALIAMTESGRTALMMSRISSGLPIFAMSRHEHTLNLTALYRGVTPVYFDSHEDGVIAANDAVNRLRDKGFLVSGDLVIVTQGDVMETVGTTNTSRILRVE

SEQ ID NO: 43 - DNA, 2137 bp, Artificial Sequence
  Synthetic DNA fragment
ttggttgaacgctttttggcttaatggccttttgaacaccacaacactgaggaaaatgaaatgaaaacaaaaagtagcctggttttattgctgccactggcgttaagtttcgcggcctttggtggagagttcagcggcaaagtcattaagctgggcgtcgaccccacctatccgccgttggaatacaagactccacagggtgcgctgaccggattcggtgtcgatattgcgcaggcaatgtgcgatcaaatgcaggccaaatgcatttgggtcgaaagcagttgggatgggatgatcccggggttgcaggcaaaaaagtttgacgccattgcctcgtccatgaccattacgccgcagcgtcaggcgcaaatagccttctcggataaagtgtccaatgccccggcacggttggtagcccgtaaaggcagcgatctgcaacctaccgcggcttcgctgaaaggcaaatccgttggcgtacaacagggatccagccaggaagcttacgccaacgcgctatggcgaccagctggggtcaatgtggtgtcctaccaaagccagcaggaagccaatgaagatttggtcaatggacggttggatgcgtcactgttggccagtgtcagcgccagtgagtttttccatacgcctgccgggaaggattttgcctttaccggtgctgagctcaatgacagcaaatatttcggtatcggcgacggtattgggttgcgtaaagaggatacggcattgctcaatgcatttaatgccgcgctgaaagcgatcatcgccaacggcacttataagaaagtgaacgataaatactttgattttgacgtgtatggttcagggcaataacggcggattggcgggaaacaaaaaataaaagggccaggcaaatgcccggcccgataaaaacggttacttcacttcgcccatagctttcagctttttggacagttcgcgacgttctttagacagatcgacatttttgatgatgtagtcatcaacgcgatcttcatagtcgctgcgcatgttgccaatgatgccctgaacgtcttcaatgctcatgcctggcttgatgtactcactcaggttgtcgagtagcagcacacgcttttggttatcacgaactttcttttcgttgtcgataatttcgcgttgcagcttatttttacggcggaacatacgcacaaactccagaacgtcctggaaactcggcttatttgcattatccatcttcatacccttgctttagtaatacacagattcatttgcttacggccacaatgataccaagatacaggtttgtggcggtcaggcacaacactcatcgccctatcttactcactttgctgtccggacaaaaacccgaagcgcctgcttcatgatctgaccccctattcgcgcccggtagcagtacagaccttgagcaggtcgcccagttcttccagttgttgtgtcagctccatgctcagccagacataaccgtaaattggcgcttcgccgtgctgactgacactggcttcctgcatcagcgttttcagttcagcggcgatttcgcttagctcgcctgccacgacagattgttgcgcttgtgggccattacgcatcgtgtccgccaatgattcaagcgaccgcagcgtcagcaattgcgcactgcgcagggttttcgcattcagcataatgaaatgggtttcacgcgaggcccaataagcgtccgccaacagctccagagtacagaccagattgcggctcaacgtttgtaccgcttcaaatacagccggaggaatatgggtttctttactgctgggaacaatcaggccgcgcaatttgaccacctgattcaagagatctttcaactgcggttccaaccgcggccgctctatcatgttcggtgacaaataagcaccgtagattttactcgcgctttgcaagcaatccgccatctgcatacgccacagaatgtaggcgcgctgagggtaaatgctggtgaacaacaacgccagcaacgaaccaaaaattacgtcaccactgcgccacaacgcggtatgcatgtcacctgcccccgcgccacaaaccaccgccagtgtaatccccaccaacagtgccatatagggccgcttaccgagtgtcagatagccgc

SEQ ID NO: 44 - protein, 109 aa, Artificial Sequence
  Synthetic peptide
METTKPSFQDVLEFVRLFRRKNKLQREIQDVEKKIRDNQKRVLLLDNLSDYIKPGMSVEAIQGIIASMKGDYEDRVDDYIIKNVELSKERRDISKKLKAMGEMKNGEAK

SEQ ID NO: 45 - DNA, 4301 bp, Artificial Sequence
  Synthetic DNA fragment
tgctggagttgcaaatcaatgcatactgggccacgcgccccagccatttcgtgttattgaacgcgcaaaaacttcgtgatacccagcacatgatgcagcaaatactgctgagccttgttcatgcgctgtacgaaggtaatccgcagccggtttttgccaatacggaaaaattgaacgatgctgtggaagagctgcgtcagttgctcaataaccaccatgacctgaaggttgtggaaacaccaatctatggttatgtgtggctgaacatggaaacggcgcatcagcttgagttgctatcgaatctgatttgccgggccttgcgcaaataattcctgaacttcagaatcatcttgctgctgcttcgattcagcaaggataaagggtatgatagtgaaaagggataaaagcattgtcatctgcggcagctatgagtaatgttggccctaacgaatagcggttgcttaaacgaatccgactctcacattatcaggggtataaaagatcctttttaacccatcacatatacctgccgttcactattatttagtgaaatgagatattatgatattttctgaattgtgattaaaaaggcaactttatgcccatgcaacagaaactataaaaaatacagagaatgaaaagaaacagatagattttttagttctttaggcccgtagtctgcaaatccttttatgattttctatcaaacaaaagaggaaaatagaccagttgcaatccaaacgagagtctaatagaatgaggtcgaaaagtaaatcgcgcgggtttgttactgataaagcaggcaagacctaaaatgtgtaaagggcaaagtgtatactttggcgtcaccccttacatattttaggtctttttttattgtgcgtaactaacttgccatcttcaaacaggagggctggaagaagcagaccgctaacacagtacataaaaaaggagacatgaacgatgaacatcaaaaagtttgcaaaacaagcaacagtattaacctttactaccgcactgctggcaggaggcgcaactcaagcgtttgcgaaagaaacgaaccaaaagccatataaggaaacatacggcatttcccatattacacgccatgatatgctgcaaatccctgaacagcaaaaaaatgaaaaatatcaagttcctgaattcgattcgtccacaattaaaaatatctcttctgcaaaaggcctggacgtttgggacagctggccattacaaaacgctgacggcactgtcgcaaactatcacggctaccacatcgtctttgcattagccggagatcctaaaaatgcggatgacacatcgatttacatgttctatcaaaaagtcggcgaaacttctattgacagctggaaaaacgctggccgcgtctttaaagacagcgacaaattcgatgcaaatgattctatcctaaaagaccaaacacaagaatggtcaggttcagccacatttacatctgacggaaaaatccgtttattctacactgatttctccggtaaacattacggcaaacaaacactgacaactgcacaagttaacgtatcagcatcagacagctctttgaacatcaacggtgtagaggattataaatcaatctttgacggtgacggaaaaacgtatcaaaatgtacagcagttcatcgatgaaggcaactacagctcaggcgacaaccatacgctgagagatcctcactacgtagaagataaaggccacaaatacttagtatttgaagcaaacactggaactgaagatggctaccaaggcgaagaatctttatttaacaaagcatactatggcaaaagcacatcattcttccgtcaagaaagtcaaaaacttctgcaaagcgataaaaaacgcacggctgagttagcaaacggcgctctcggtatgattgagctaaacgatgattacacactgaaaaaagtgatgaaaccgctgattgcatctaacacagtaacagatgaaattgaacgcgcgaacgtctttaaaatgaacggcaaatggtacctgttcactgactcccgcggatcaaaaatgacgattgacggcattacgtctaacgatatttacatgcttggttatgtttctaattctttaactggcccatacaagccgctgaacaaaactggccttgtgttaaaaatggatcttgatcctaacgatgtaacctttacttactcacacttcgctgtacctcaagcgaaaggaaacaatgtcgtgattacaagctatatgacaaacagaggattctacgcagacaaacaatcaacgtttgcgccaagcttcctgctgaacatcaaaggcaagaaaacatctgttgtcaaagacagcatccttgaacaaggacaattaacagttaacaaataaaaacgcaaaagaaaatgccgatatcctattggcattttcttttatttcttatcaacataaaggtgaatcccatatgaactatataaaagcaggcaaatggctaaccgtattcctaacctttttaggaatattgctgtttatcgacttgtcgactctagaggatcctgtgtaggctggagctgcttcgaagttcctatactttctagagaataggaacttcggaataggaacttcaagatcccctcacgctgccgcaagcactcagggcgcaagggctgctaaaggaagcggaacacgtagaaagccagtccgcagaaacggtgctgaccccggatgaatgtcagctactgggctatctggacaagggaaaacgcaagcgcaaagagaaagcaggtagcttgcagtgggcttacatggcgatagctagactgggcggttttatggacagcaagcgaaccggaattgccagctggggcgccctctggtaaggttgggaagccctgcaaagtaaactggatggctttcttgccgccaaggatctgatggcgcaggggatcaagatctgatcaagagacaggatgaggatcgtttcgcatgattgaacaagatggattgcacgcaggttctccggccgcttgggtggagaggctattcggctatgactgggcacaacagacaatcggctgctctgatgccgccgtgttccggctgtcagcgcaggggcgcccggttctttttgtcaagaccgacctgtccggtgccctgaatgaactgcaggacgaggcagcgcggctatcgtggctggccacgacgggcgttccttgcgcagctgtgctcgacgttgtcactgaagcgggaagggactggctgctattgggcgaagtgccggggcaggatctcctgtcatctcaccttgctcctgccgagaaagtatccatcatggctgatgcaatgcggcggctgcatacgcttgatccggctacctgcccattcgaccaccaagcgaaacatcgcatcgagcgagcacgtactcggatggaagccggtcttgtcgatcaggatgatctggacgaagagcatcaggggctcgcgccagccgaactgttcgccaggctcaaggcgcgcatgcccgacggcgaggatctcgtcgtgacccatggcgatgcctgcttgccgaatatcatggtggaaaatggccgcttttctggattcatcgactgtggccggctgggtgtggcggaccgctatcaggacatagcgttggctacccgtgatattgctgaagagcttggcggcgaatgggctgaccgcttcctcgtgctttacggtatcgccgctcccgattcgcagcgcatcgccttctatcgccttcttgacgagttcttctgagcgggactctggggttcgaaatgaccgttcccgttttattcaatgagggttgcccggcaaccctcattgctcattgattcttatctgtgtatcaccgtcatcattctcatccgagaaccaatcgaaattaacaacagccttcttctgtatgcagcaaggcaaaaagttctgtaactccattgttattaactgcactggttactaacacgttgtgcgctccagcttcccgtaaccaacttttcaccaaagatatttgttccatgctggctaaatctgctttggttactactccaatgaccgggtgattcatggcccggtagggcgtttttacctctaattcctgcttcagcgctgagattcctgcttgttgccagaaaagcaggcacctgccgtctgaacggtatcgatccggaagcgtatctgcgccatattctgagcatactgccggaatggccctccaaccgtgttgacgaactcctgccatggaacgtagttctcaccaataaataagcgtcaatacggtgctc

SEQ ID NO: 46 - DNA, 22 bp, Artificial Sequence
  Primer
tgctggagttgcaaatcaatgc

SEQ ID NO: 47 - DNA, 22 bp, Artificial Sequence
  Primer
gagcaccgtattgacgcttatt

SEQ ID NO: 48 - DNA, 1330 bp, Artificial Sequence
  Synthetic DNA fragment
tgctggagttgcaaatcaatgcatactgggccacgcgccccagccatttcgtgttattgaacgcgcaaaaacttcgtgatacccagcacatgatgcagcaaatactgctgagccttgttcatgcgctgtacgaaggtaatccgcagccggtttttgccaatacggaaaaattgaacgatgctgtggaagagctgcgtcagttgctcaataaccaccatgacctgaaggttgtggaaacaccaatctatggttatgtgtggctgaacatggaaacggcgcatcagcttgagttgctatcgaatctgatttgccgggccttgcgcaaataattcctgaacttcagaatcatcttgctgctgcttcgattcagcaaggataaagggtatgatagtgaaaagggataaaagcattgtcatctgcggcagctatgagtaatgttggccctaacgaatagcggttgcttaaacgaatccgactctcacattatcaggggtataaaaatggaaactaccaagccttcattccaggacgtactggaatttgttcgtctgttccgtcgtaagaacaaactgcaacgtgaaattcaggacgttgagaaaaagatccgtgacaaccagaagcgcgtcctgctgctggacaacctgagcgattacatcaagccggggatgagcgttgaagcaatccagggcatcatcgccagcatgaaaggtgactatgaagatcgcgttgacgattacatcatcaaaaatgccgagctctccaaagaacgccgcgatatctccaaaaagctgaaagctatgggcgaaatgaaaaacggcgaagcgaagtaattcccgttttattcaatgagggttgcccggcaaccctcattgctcattgattcttatctgtgtatcaccgtcatcattctcatccgagaaccaatcgaaattaacaacagccttcttctgtatgcagcaaggcaaaaagttctgtaactccattgttattaactgcactggttactaacacgttgtgcgctccagcttcccgtaaccaacttttcaccaaagatatttgttccatgctggctaaatctgctttggttactactccaatgaccgggtgattcatggcccggtagggcgtttttacctctaattcctgcttcagcgctgagattcctgcttgttgccagaaaagcaggcacctgccgtctgaacggtatcgatccggaagcgtatctgcgccatattctgagcatactgccggaatggccctccaaccgtgttgacgaactcctgccatggaacgtagttctcaccaataaataagcgtcaatacggtgctc

SEQ ID NO: 49 - DNA, 42 bp, Artificial Sequence
  Primer
accaccatcacgtgggtacctgctggagttgcaaatcaatgc

SEQ ID NO: 50 - DNA, 42 bp, Artificial Sequence
  Primer
cgtcgtcatcattcgaaccggagcaccgtattgacgcttatt